European Patent Application EP 4 516 905 A1, published March 5, 2025. Title: 心外膜細胞再生促進剤および心外膜細胞の再生促進方法. Applicant: 国立大学法人京都大学. Application JP. The sequence listing filed with the application follows.

SEQUENCE LISTING (10 sequences)

SEQ ID NO: 1 - RNA, 21 nt, synthetic construct
  source 1..21: mol_type = other RNA
  modified_base 20..21: mod_base = OTHER; note = thymine
caaggagtcagacattttatt

SEQ ID NO: 2 - RNA, 21 nt, synthetic construct
  source 1..21: mol_type = other RNA
  modified_base 20..21: mod_base = OTHER; note = thymine
taaaatgtctgactccttgtt

SEQ ID NO: 3 - DNA, 18 bp, synthetic construct
  misc_feature 1..18: note = primer
  source 1..18: mol_type = other DNA
aggggacagcagaggaag

SEQ ID NO: 4 - DNA, 23 bp, synthetic construct
  misc_feature 1..23: note = primer
  source 1..23: mol_type = other DNA
gcgtttggagtggtagaaatctg

SEQ ID NO: 5 - DNA, 20 bp, synthetic construct
  misc_feature 1..20: note = primer
  source 1..20: mol_type = other DNA
cagcttgaatgcatgacctg

SEQ ID NO: 6 - DNA, 20 bp, synthetic construct
  misc_feature 1..20: note = primer
  source 1..20: mol_type = other DNA
gatgccgaccgtacaagagt

SEQ ID NO: 7 - DNA, 25 bp, synthetic construct
  misc_feature 1..25: note = primer
  source 1..25: mol_type = other DNA
tgatgacatcaagaaggtggtgaag

SEQ ID NO: 8 - DNA, 22 bp, synthetic construct
  misc_feature 1..22: note = primer
  source 1..22: mol_type = other DNA
tccttggaggccatgtggccat

SEQ ID NO: 9 - DNA, 2126 bp, synthetic construct
  misc_feature 1..2126: note = Synthetic
  source 1..2126: mol_type = other DNA
atgttgagctctggcatagaagaggctggtggctattttgtccttgggctgcctgttttcagctgctgcaaccacagggatttcttctgttcaggcgccatgtcagaaccggctggggatgtccgtcagaacccatgcggcagcaaggcctgccgccgcctcttcggcccagtggacagcgagcagctgagccgcgactgtgatgcgctaatggcgggctgcatccaggaggcccgtgagcgatggaacttcgactttgtcaccgagacaccactggagggtgacttcgcctgggagcgtgtgcggggccttggcctgcccaagctctaccttcccacggggccccggcgaggccgggatgagttgggaggaggcaggcggcctggcacctcacctgctctgctgcaggggacagcagaggaagaccatgtggacctgtcactgtcttgtacccttgtgcctcgctcaggggagcaggctgaagggtccccaggtggacctggagactctcagggtcgaaaacggcggcagaccagcatgacagatttctaccactccaaacgccggctgatcttctccaagaggaagccctaatccgcccacaggaagcctgcagtcctggaagcgcgagggcctcaaaggcccgctctacatcttctgccttagtctcagtttgtgtgtcttaattattatttgtgttttaatttaaacacctcctcatgtacataccctggccgccccctgccccccagcctctggcattagaattatttaaacaaaaactaggcggttgaatgagaggttcctaagagtgctgggcatttttattttatgaaatactatttaaagcctcctcatcccgtgttctccttttcctctctcccggaggttgggtgggccggcttcatgccagctacttcctcctccccacttgtccgctgggtggtaccctctggaggggtgtggctccttcccatcgctgtcacaggcggttatgaaattcaccccctttcctggacactcagacctgaattctttttcatttgagaagtaaacagatggcactttgaaggggcctcaccgagtgggggcatcatcaaaaactttggagtcccctcacctcctctaaggttgggcagggtgaccctgaagtgagcacagcctagggctgagctggggacctggtaccctcctggctcttgatacccccctctgtcttgtgaaggcagggggaaggtggggtcctggagcagaccaccccgcctgccctcatggcccctctgacctgcactggggagcccgtctcagtgttgagccttttccctctttggctcccctgtaccttttgaggagccccagctaccctttttctccagctgggctctgcaattcccctctgctgctgtccctcccccttgtcctttcccttcagtaccctctcagctccaggtggctctgaggtgcctgtcccacccccacccccagctcaatggactggaaggggaagggacacacaagaagaagggcaccctagttctacctcaggcagctcaagcagcgaccgccccctcctctagctgtgggggtgagggtcccatgtggtggcacaggcccccttgagtggggttatctctgtgttaggggtatatgatgggggagtagatctttctaggagggagacactggcccctcaaatcgtccagcgaccttcctcatccaccccatccctccccagttcattgcactttgattagcagcggaacaaggagtcagacattttaagatggtggcagtagaggctatggacagggcatgccacgtgggctcatatggggctgggagtagttgtctttcctggcactaacgttgagcccctggaggcactgaagtgcttagtgtacttggagtattggggtctgaccccaaacaccttccagctcctgtaacatactggcctggactgttttctctcggctccccatgtgtcctggttcccgtttctccacctagactgtaaacctctcgagggcagggaccacaccctgtactgttctgtgtctttcacagctcctcccacaatgctgaatatacagcaggtgctcaataaatgattcttagtgacttta

SEQ ID NO: 10 - protein, 164 aa, synthetic construct
  REGION 1..164: note = Synthetic
MSEPAGDVRQNPCGSKACRRLFGPVDSEQLSRDCDALMAGCIQEARERWNFDFVTETPLEGDFAWERVRGLGLPKLYLPTGPRRGRDELGGGRRPGTSPALLQGTAEEDHVDLSLSCTLVPRSGEQAEGSPGGPGDSQGRKRRQTSMTDFYHSKRRLIFSKRKP